European Patent Application EP 4 332 113 A1, published March 6, 2024. Title: Novel regulators of acetate metabolism A variant and a method for producing L-brached chain amino acids using the same. Applicant: CJ CheilJedang Corporation. The sequence listing filed with the application follows.

SEQUENCE LISTING (16 sequences)

SEQ ID NO: 1 - protein, 281 aa, synthetic construct
  REGION 1..281: note = regulators of acetate metabolism A variant (L56A)
VDTQRIKDDEDAIRSALTSLKTATGIPVTMFATVLQDNRLQITQWVGLRTPALQNAVIEPGVGVGGRVVATRRPVGVSDYTRANVISHEKDSAIQDEGLHSIVAVPVIVHREIRGVLYVGVHSAVRLGDTVIEEVTMTARTLEQNLAINSALRRNGVPDGRGSLKASRVMNGAEWEQVRSTHSKLRMLANRVTDEDLRRDLEELCDQMVTPVRIKQTTKLSARELDVLACVALGHTNVEAAEEMGIGAETVKSYLRSVMRKLGAHTRYEAVNAARRIGALP

SEQ ID NO: 2 - DNA, 846 bp, synthetic construct
  misc_feature 1..846: note = regulators of acetate metabolism A variant (L56A)
  source 1..846: mol_type = other DNA
gtggatacccagcggattaaagatgacgaagatgctattcgttcggcgctgacatcgctgaaaaccgcaacaggcatcccagtcaccatgttcgccactgtgttgcaggacaatcgcctgcaaattactcagtgggttgggttgcgtaccccggctctgcagaatgcggtcattgaaccaggtgtgggcgttggtggacgcgtcgtcgcaacccgtcgtccggttggtgtgagtgattacaccagggcaaatgtcatttcacatgagaaggattccgcgattcaggatgagggccttcattccattgtcgcagttcccgtgatcgtgcaccgcgaaatccgtggcgttttgtatgttggcgttcactctgcggtgcgtctcggcgacactgttattgaagaagtcaccatgactgcgcgcacgttggaacaaaacctggcgatcaactccgcgcttcgccgcaatggcgttcctgatggtcgcggttccctcaaagctagccgcgtgatgaatggggcggagtgggagcaggttcgttccactcattccaagctgcgcatgctggcaaatcgtgtgaccgatgaggatctgcgccgcgatttggaagagctttgcgatcagatggtcaccccagtccgcatcaagcagaccaccaagctgtccgcgcgtgagttggacgtgctggcttgtgtcgcgctcggtcacaccaacgtcgaagctgctgaagagatgggcatcggcgcggaaaccgtcaagagctacctgcgctcggtcatgcgcaagctcggcgcccacacgcgctacgaggcagtcaacgcagcacgccggatcggcgcactgccttaa

SEQ ID NO: 3 - protein, 281 aa, unidentified
  REGION 1..281: note = regulators of acetate metabolism A
VDTQRIKDDEDAIRSALTSLKTATGIPVTMFATVLQDNRLQITQWVGLRTPALQNLVIEPGVGVGGRVVATRRPVGVSDYTRANVISHEKDSAIQDEGLHSIVAVPVIVHREIRGVLYVGVHSAVRLGDTVIEEVTMTARTLEQNLAINSALRRNGVPDGRGSLKASRVMNGAEWEQVRSTHSKLRMLANRVTDEDLRRDLEELCDQMVTPVRIKQTTKLSARELDVLACVALGHTNVEAAEEMGIGAETVKSYLRSVMRKLGAHTRYEAVNAARRIGALP

SEQ ID NO: 4 - DNA, 846 bp, unidentified
  misc_feature 1..846: note = regulators of acetate metabolism A
  source 1..846: mol_type = genomic DNA
gtggatacccagcggattaaagatgacgaagatgctattcgttcggcgctgacatcgctgaaaaccgcaacaggcatcccagtcaccatgttcgccactgtgttgcaggacaatcgcctgcaaattactcagtgggttgggttgcgtaccccggctctgcagaatctggtcattgaaccaggtgtgggcgttggtggacgcgtcgtcgcaacccgtcgtccggttggtgtgagtgattacaccagggcaaatgtcatttcacatgagaaggattccgcgattcaggatgagggccttcattccattgtcgcagttcccgtgatcgtgcaccgcgaaatccgtggcgttttgtatgttggcgttcactctgcggtgcgtctcggcgacactgttattgaagaagtcaccatgactgcgcgcacgttggaacaaaacctggcgatcaactccgcgcttcgccgcaatggcgttcctgatggtcgcggttccctcaaagctagccgcgtgatgaatggggcggagtgggagcaggttcgttccactcattccaagctgcgcatgctggcaaatcgtgtgaccgatgaggatctgcgccgcgatttggaagagctttgcgatcagatggtcaccccagtccgcatcaagcagaccaccaagctgtccgcgcgtgagttggacgtgctggcttgtgtcgcgctcggtcacaccaacgtcgaagctgctgaagagatgggcatcggcgcggaaaccgtcaagagctacctgcgctcggtcatgcgcaagctcggcgcccacacgcgctacgaggcagtcaacgcagcacgccggatcggcgcactgccttaa

SEQ ID NO: 5 - protein, 281 aa, synthetic construct
  REGION 1..281: note = regulators of acetate metabolism A variant (L56A+A52V)
VDTQRIKDDEDAIRSALTSLKTATGIPVTMFATVLQDNRLQITQWVGLRTPVLQNAVIEPGVGVGGRVVATRRPVGVSDYTRANVISHEKDSAIQDEGLHSIVAVPVIVHREIRGVLYVGVHSAVRLGDTVIEEVTMTARTLEQNLAINSALRRNGVPDGRGSLKASRVMNGAEWEQVRSTHSKLRMLANRVTDEDLRRDLEELCDQMVTPVRIKQTTKLSARELDVLACVALGHTNVEAAEEMGIGAETVKSYLRSVMRKLGAHTRYEAVNAARRIGALP

SEQ ID NO: 6 - DNA, 846 bp, synthetic construct
  misc_feature 1..846: note = regulators of acetate metabolism A variant (L56A+A52V)
  source 1..846: mol_type = other DNA
gtggatacccagcggattaaagatgacgaagatgctattcgttcggcgctgacatcgctgaaaaccgcaacaggcatcccagtcaccatgttcgccactgtgttgcaggacaatcgcctgcaaattactcagtgggttgggttgcgtaccccggttctgcagaatgcggtcattgaaccaggtgtgggcgttggtggacgcgtcgtcgcaacccgtcgtccggttggtgtgagtgattacaccagggcaaatgtcatttcacatgagaaggattccgcgattcaggatgagggccttcattccattgtcgcagttcccgtgatcgtgcaccgcgaaatccgtggcgttttgtatgttggcgttcactctgcggtgcgtctcggcgacactgttattgaagaagtcaccatgactgcgcgcacgttggaacaaaacctggcgatcaactccgcgcttcgccgcaatggcgttcctgatggtcgcggttccctcaaagctagccgcgtgatgaatggggcggagtgggagcaggttcgttccactcattccaagctgcgcatgctggcaaatcgtgtgaccgatgaggatctgcgccgcgatttggaagagctttgcgatcagatggtcaccccagtccgcatcaagcagaccaccaagctgtccgcgcgtgagttggacgtgctggcttgtgtcgcgctcggtcacaccaacgtcgaagctgctgaagagatgggcatcggcgcggaaaccgtcaagagctacctgcgctcggtcatgcgcaagctcggcgcccacacgcgctacgaggcagtcaacgcagcacgccggatcggcgcactgccttaa

SEQ ID NO: 7 - DNA, 28 bp, synthetic construct
  misc_feature 1..28: note = primer
  source 1..28: mol_type = other DNA
ctattctagaatgggggtagcgggtgtg

SEQ ID NO: 8 - DNA, 27 bp, synthetic construct
  misc_feature 1..27: note = primer
  source 1..27: mol_type = other DNA
ctattctagagcggacagcttggtggt

SEQ ID NO: 9 - DNA, 31 bp, synthetic construct
  misc_feature 1..31: note = primer
  source 1..31: mol_type = other DNA
cggggatcctctagactaataccgcaaatgg

SEQ ID NO: 10 - DNA, 18 bp, synthetic construct
  misc_feature 1..18: note = primer
  source 1..18: mol_type = other DNA
tgaccagattctgcagaa

SEQ ID NO: 11 - DNA, 18 bp, synthetic construct
  misc_feature 1..18: note = primer
  source 1..18: mol_type = other DNA
ttctgcagaatctggtca

SEQ ID NO: 12 - DNA, 31 bp, synthetic construct
  misc_feature 1..31: note = primer
  source 1..31: mol_type = other DNA
caggtcgactctagaggtggtctgcttgatg

SEQ ID NO: 13 - DNA, 32 bp, synthetic construct
  misc_feature 1..32: note = primer
  source 1..32: mol_type = other DNA
aatttctagaggcagaccctattctatgaagg

SEQ ID NO: 14 - DNA, 30 bp, synthetic construct
  misc_feature 1..30: note = primer
  source 1..30: mol_type = other DNA
agtgtttcggtctttacagacacgagggac

SEQ ID NO: 15 - DNA, 30 bp, synthetic construct
  misc_feature 1..30: note = primer odhA_down_F
  source 1..30: mol_type = other DNA
gtccctcgtgtctgtaaagaccgaaacact

SEQ ID NO: 16 - DNA, 32 bp, synthetic construct
  misc_feature 1..32: note = primer
  source 1..32: mol_type = other DNA
aatttctagacgtgggagtgtcactcgcttgg